European Patent Specification EP 4 065 136 B1, published August 14, 2024. Title: Phagocytosed self-assembling proteins. Applicant: CELL GUIDANCE SYSTEMS LIMITED. The sequence listing filed with the application follows.

SEQUENCE LISTING (4 sequences)

SEQ ID NO: 1 - protein, 250 aa, Bombyx mori
MIMADVAGTSNRDFRGREQRLFNSEQYNYNSSLNGEVSVWVYAYYSDGSVLVINKNSQYKVGISETFKALKEYREGQHNDSYDEYEVNQSIYYPNGGDARKFHSNAKPRAIQIIFSPSVNVRTIKMAKGNAVSVPDEYLQRSHPWEATGIKYRKIKRDGEIVGYSHYFELPHEYNSISLAVSGVHKNPSSYNVGSAHNVMDVFQSCDLALRFCNRYWAELELVNHYISPNAYPYLDINNHSYGVALSNRQ

SEQ ID NO: 2 - protein, 30 aa, Artificial Sequence
  H1-tag
MADVAGTSNRDFRGREQRLFNSEQYNYNNS

SEQ ID NO: 3 - protein, 53 aa, Artificial Sequence
  VP3-tag
AFNSQRRSHTLRLLGPFQYFNFSETDRGHPLFRLPLKYPSKAIPADELIDNLH

SEQ ID NO: 4 - protein, 235 aa, Artificial Sequence
  PH-tag
GREQRLFNSEQYNYNSSLNGEVSVWVYAYYSDGSVLVINKNSQYKVGISETFKALKEYREGQHNDSYDEYEVNQSIYYPNGGDARKFHSNAKPRAIQIIFSPSVNVRTIKMAKGNAVSVPDEYLQRSHPWEATGIKYRKIKRDGEIVGYSHYFELPHEYNSISLAVSGVHKNPSSYNVGSAHNVMDVFQSCDLALRFCNRYWAELELVNHYISPNAYPYLDINNHSYGVALSNRQ